European Patent Application EP 4 122 950 A1, published January 25, 2023. Title: Recombinant host cells and methods for producing casein proteins. Applicant: Redbiotec AG. The sequence listing filed with the application follows.

SEQUENCE LISTING (37 sequences)

SEQ ID NO: 1 - protein, 199 aa, bovine
RPKHPIKHQGLPQEVLNENLLRFFVAPFPEVFGKEKVNELSKDIGSESTEDQAMEDIKQMEAESISSSEEIVPNSVEQKHIQKEDVPSERYLGYLEQLLRLKKYKVPQLEIVPNSAEERLHSMKEGIHAQQKEPMIGVNQELAYFYPELFRQFYQLDAYPSGAWYYVPLGTQYTDAPSFSDIPNPIGSENSEKTTMPLW

SEQ ID NO: 2 - protein, 199 aa, bovine
RPKHPIKHQGLPQEVLNENLLRFFVAPFPEVFGKEKVNELEKDIGEEETEDQAMEDIKQMEAEEIEEEEEIVPNEVEQKHIQKEDVPSERYLGYLEQLLRLKKYKVPQLEIVPNSAEERLHSMKEGIHAQQKEPMIGVNQELAYFYPELFRQFYQLDAYPSGAWYYVPLGTQYTDAPSFSDIPNPIGSENSEKTTMPLW

SEQ ID NO: 3 - DNA, 597 bp, bovine
cgaccaaaacatcctatcaagcatcaaggattgcctcaagaagtcttgaacgaaaatttactcaggttttttgtggcaccttttccagaagtctttggaaaggagaaggtcaatgaactgtccaaggacattggtagtgaatcaactgaggatcaagcaatggaagatattaagcaaatggaagctgaaagcatttcgtcatccgaggaaattgttcccaatagcgttgagcagaagcacatacaaaaggaggatgtaccgtctgagcgttacctgggttatctggagcagcttctcagattgaaaaaatacaaagtaccccagttggaaattgttcccaactctgctgaggaaagattgcactccatgaaagagggaatccatgcgcaacagaaagaacctatgataggtgtgaaccaggaacttgcctacttctatcctgagcttttcagacaattctaccaactggatgcctatccatctggtgcatggtattacgttccactagggacacaatataccgacgccccatcattctctgacatcccaaatcctattggctctgagaacagtgaaaagactacgatgccattgtgg

SEQ ID NO: 4 - DNA, 597 bp, bovine
agaccaaaacatcctataaagcatcaaggtttgcctcaagaagtcttgaacgaaaatttactcaggttttttgtagcaccatttccagaagtgtttggaaaggagaaggtcaacgaactgagcaaggatataggggaagaagagactgaggatcaagcaatggaagatattaagcaaatggaggctgaagagattgaagaggaagaggaaattgttcctaatgaggttgagcaaaagcacattcaaaaggaagatgtgccctccgagcgttatttaggttatttggagcagctattgagattgaaaaaatacaaagtaccccagctggaaattgttcccaatgaagctgaggaacgacttcactccatgaaagagggaatccatgcacaacagaaagaaccgatgataggagtcaaccaggaactggcctacttctaccctgagttgttcagacaattctaccagctggacgcctatccatctggtgcctggtattacgttccactaggtacacaatatactgacgcgccatcattctctgacatccctaatcctattggctcggagaacagtgaaaagacgaccatgccactttgg

SEQ ID NO: 5 - protein, 207 aa, bovine
KNTMEHVSSSEESIISQETYKQEKNMAINPSKENLCSTFCKEVVRNANEEEYSIGSSSEESAEVATEEVKITVDDKHYQKALNEINQFYQKFPQYLQYLYQGPIVLNPWDQVKRNAVPITPTLNREQLSTSEENSKKTVDMESTEVFTKKTKLTEEEKNRLNFLKKISQRYQKFALPQYLKTVYQHQKAMKPWIQPKTKVIPYVRYL

SEQ ID NO: 6 - protein, 207 aa, bovine
KNTMEHVEEEEESIIEQETYKQEKNMAINPEKENLCSTFCKEVVRNANEEEYSIGEEEEEEAEVATEEVKITVDDKHYQKALNEINQFYQKFPQYLQYLYQGPIVLNPWDQVKRNAVPITPTLNREQLETEEENSKKTVDMEETEVFTKKTKLTEEEKNRLNFLKKISQRYQKFALPQYLKTVYQHQKAMKPWIQPKTKVIPYVRYL

SEQ ID NO: 7 - DNA, 621 bp, bovine
aagaacacgatggaacatgtctcctctagtgaggagtctataatctcgcaagagacatacaagcaggagaagaatatggccattaatccaagcaaggagaacttgtgttccaccttctgcaaggaagtcgtaaggaacgcaaatgaagaggaatactctatcggatcatctagtgaggaatctgctgaggttgccactgaggaagtcaagattactgtggacgataagcactaccaaaaagctctaaacgaaatcaatcagttttatcaaaagtttccccaatatttgcaatatctgtaccaaggtccaattgttttgaacccttgggatcaggttaaaagaaatgctgttccgattactccaactttaaacagagagcaactctccaccagtgaggaaaattcaaaaaaaaccgtggacatggaatcaacagaagtattcactaagaaaacaaaactgacggaagaagaaaagaacagactaaattttttaaaaaaaatcagccaacgttaccagaaatttgcgttgccacagtatctgaaaactgtctatcagcatcaaaaagctatgaagccttggattcaacctaagacaaaggttattccctatgtgcgatacctt

SEQ ID NO: 8 - DNA, 621 bp, bovine
aagaatacgatggaacatgtcgaagaggaagaggagtctatcatagagcaagaaacatacaaacaggaaaagaatatggcgattaatccggaaaaagagaacctttgctccacattctgtaaggaagtcgtaaggaacgcaaatgaggaggagtattctataggagaagaggaagaggaagaggctgaagtcgccacggaggaagttaagattactgtggacgataagcactaccaaaaagcacttaacgaaatcaatcaattttaccaaaagttcccacagtatttacaatacctgtatcaaggtccaattgtcttgaacccctgggatcaagttaagagaaatgctgttccaattaccccaactctgaacagagagcagttggaaaccgaagaggaaaactcaaaaaagaccgttgacatggaagagacagaggtattcactaagaaaactaaattgactgaagaagaaaagaaccgactaaattttctgaaaaaaatcagtcaacgttaccagaaattcgccttgccccagtatctcaagactgtgtatcaacatcagaaagctatgaaaccttggattcaacctaaaacaaaggttattccttatgtgagataccta

SEQ ID NO: 9 - protein, 209 aa, bovine
RELEELNVPGEIVESLSSSEESITRINKKIEKFQSEEQQQTEDELQDKIHPFAQTQSLVYPFPGPIPNSLPQNIPPLTQTPVVVPPFLQPEVMGVSKVKEAMAPKHKEMPFPKYPVEPFTESQSLTLTDVENLHLPLPLLQSWMHQPHQPLPPTVMFPPQSVLSLSQSKVLPVPQKAVPYPQRDMPIQAFLLYQEPVLGPVRGPFPIIV

SEQ ID NO: 10 - protein, 209 aa, bovine
RELEELNVPGEIVEELEEEEESITRINKKIEKFQEEEQQQTEDELQDKIHPFAQTQSLVYPFPGPIPNSLPQNIPPLTQTPVVVPPFLQPEVMGVSKVKEAMAPKHKEMPFPKYPVEPFTESQSLTLTDVENLHLPLPLLQSWMHQPHQPLPPTVMFPPQSVLSLSQSKVLPVPQKAVPYPQRDMPIQAFLLYQEPVLGPVRGPFPIIV

SEQ ID NO: 11 - DNA, 627 bp, bovine
agagagttggaagaattaaatgtaccaggtgagatagttgaatctctatcaagctcggaggaatcaattacccgtataaacaagaaaattgagaagtttcagagtgaggaacaacagcaaacagaggacgaattgcaagataaaatccatccatttgcgcaaacacagtctctagtctatcccttccctggaccgatccctaactcactcccacaaaacattcctcctttaactcaaacccctgtggttgttccgccattcttgcaaccagaagtaatgggagtttccaaagttaaggaggctatggctcctaagcataaggaaatgcccttcccaaaatatccagttgagccctttactgaaagccagtctctgactcttacggacgttgaaaatttgcaccttccactaccattgttgcagtcttggatgcatcaacctcaccaacctttaccaccaactgtcatgtttcctcctcaatccgtgttgagtctttctcagtccaaagtcttgcctgttccgcagaaagctgtgccatacccacagagagatatgcccattcaagcatttttgctgtaccaagaaccagtattaggtccagttaggggccccttccctattattgtc

SEQ ID NO: 12 - DNA, 627 bp, bovine
agagagttggaagaattaaatgtaccaggtgagatagttgaagagctagaagaggaagaggaatcaattacccgtataaacaagaaaattgagaagtttcaggaagaggaacaacagcaaacagaggacgaattgcaagataaaatccatccatttgcgcaaacacagtctctagtctatcccttccctggaccgatccctaactcactcccacaaaacattcctcctttaactcaaacccctgtggttgttccgccattcttgcaaccagaagtaatgggagtttccaaagttaaggaggctatggctcctaagcataaggaaatgcccttcccaaaatatccagttgagccctttactgaaagccagtctctgactcttacggacgttgaaaatttgcaccttccactaccattgttgcagtcttggatgcatcaacctcaccaacctttaccaccaactgtcatgtttcctcctcaatccgtgttgagtctttctcagtccaaagtcttgcctgttccgcagaaagctgtgccatacccacagagagatatgcccattcaagcatttttgctgtaccaagaaccagtattaggtccagttaggggccccttccctattattgtc

SEQ ID NO: 13 - protein, 168 aa, bovine
EQNQEQPIRCEKDERFFSDKIAKYIPIQYVLSRYPSYGLNYYQQKPVALINNQFLPYPYYAKPAAVRSPAQILQWQVLSNTVPAKSCQAQPTTMARHPHPHLSFMAIPPKKNQDKTEIPTINTIASGEPTSTPTIEAVESTVATLEASPEVIESPPEINTVQVTSTAV

SEQ ID NO: 14 - protein, 168 aa, bovine
EQNQEQPIRCEKDERFFSDKIAKYIPIQYVLSRYPSYGLNYYQQKPVALINNQFLPYPYYAKPAAVRSPAQILQWQVLSNTVPAKSCQAQPTTMARHPHPHLSFMAIPPKKNQDKTEIPTINTIAEGEPTSTPTIEAVESTVAELEAEPEVIESPPEINTVQVTSTAV

SEQ ID NO: 15 - DNA, 507 bp, bovine
gaacaaaaccaagaacaacccataagatgtgagaaggatgaaagattcttctctgacaaaatagccaaatatataccaattcagtacgtgctatctaggtatcctagctatggactcaattactaccaacagaaaccagttgctttgattaacaatcaatttcttccatacccctattacgcaaagcccgctgcagttcgatcccctgcgcaaattcttcaatggcaagtcttgtcaaatactgtgcctgctaagtcctgccaagctcagccgacgacgatggctcgtcacccacatccacatttatcttttatggccattccgccaaagaaaaatcaggataaaacagaaatccctaccatcaacaccattgctagtggcgagcctacatccacacctaccattgaagcagtagagtcaactgtagctactttggaagcctctccagaagttattgagtcgccacctgagatcaacacagtccaggttacttcaactgctgtctaa

SEQ ID NO: 16 - DNA, 507 bp, bovine
gaacaaaaccaagaacaaccaatacgatgtgagaaagatgaaagattcttctcggacaaaatagctaaatatatcccaattcagtatgtgctttctaggtatcctagttatggactcaattactaccaacagaaacccgttgcgctaattaacaatcagtttttgccctacccatactacgctaagccagctgcagttagatcacctgcccaaattcttcaatggcaagtcttgtcaaatactgtgcctgccaagtcctgccaagctcagccgactacaatggctcgtcacccgcatccacatttatcttttatggctattccaccaaagaagaaccaggataaaacggaaatacctaccatcaataccattgctgaaggcgagcctacatctacacctacgattgaagcagtagagagcactgtagctgagttggaagccgagccagaagttattgagtccccccctgagatcaacaccgtccaagttacttctactgcagtctaa

SEQ ID NO: 17 - protein, 185 aa, human
MRLLILTCLVAVALARPKLPLRYPERLQNPSESSEPIPLESREEYMNGMNRQRNILREKQTDEIKDTRNESTQNCVVAEPEKMESSISSSSEEMSLSKCAEQFCRLNEYNQLQLQAAHAQEQIRRMNENSHVQVPFQQLNQLAAYPYAVWYYPQIMQYVPFPPFSDISNPTAHENYEKNNVMLQW

SEQ ID NO: 18 - protein, 226 aa, human
MKVLILACLVALALARETIESLSSSEESITEYKQKVEKVKHEDQQQGEDEHQDKIYPSFQPQPLIYPFVEPIPYGFLPQNILPLAQPAVVLPVPQPEIMEVPKAKDTVYTKGRVMPVLKSPTIPFFDPQIPKLTDLENLHLPLPLLQPLMQQVPQPIPQTLALPPQPLWSVPQPKVLPIPQQVVPYPQRAVPVQALLLNQELLLNPTHQIYPVTQPLAPVHNPISV

SEQ ID NO: 19 - protein, 182 aa, human
MKSFLLVVNALALTLPFLAVEVQNQKQPACHENDERPFYQKTAPYVPMYYVPNSYPYYGTNLYQRRPAIAINNPYVPRTYYANPAVVRPHAQIPQRQYLPNSHPPTVVRRPNLHPSFIAIPPKKIQDKIIIPTINTIATVEPTPAPATEPTVDSVVTPEAFSESIITSTPETTTVAVTPPTA

SEQ ID NO: 20 - DNA, 558 bp, human
atgaggcttctcattctcacctgtcttgtggctgttgctcttgccaggcctaaacttcctcttagatacccagaacgccttcagaatccatcagagagcagtgagcctataccattagaatcaagagaggaatacatgaatggtatgaacaggcagagaaacattctgagagaaaaacagactgatgaaatcaaggatactaggaatgagtctactcagaactgtgttgtggcagagcctgagaagatggaatccagcatcagttcatcgagtgaggaaatgtctctcagtaagtgtgcggaacagttttgtagactgaacgaatacaaccaacttcagctgcaagctgcccatgcccaggagcaaattcgcagaatgaatgaaaacagccatgtccaagtgcctttccagcagctcaaccaacttgctgcctacccctatgctgtttggtactatccacaaatcatgcagtatgttcctttcccaccgttttccgacatctccaatcccactgctcatgaaaattatgaaaaaaataacgtcatgctacagtggtga

SEQ ID NO: 21 - DNA, 681 bp, human
atgaaggtcctcatcctcgcctgcctggtggctcttgctcttgcaagggagaccatagaaagcctttcaagcagtgaggaatctattacagaatacaagcagaaagttgagaaggttaaacatgaggaccagcagcaaggagaggatgaacaccaggataaaatctacccctctttccagccacagcctctgatctatccattcgttgaacctatcccctatggttttcttccacaaaacattctgcctcttgctcagcctgctgtggtgctgcctgtccctcagcctgaaataatggaagtccctaaagctaaagacactgtctacactaagggcagagtgatgcctgtccttaaatctccaacgatacccttttttgaccctcaaatcccaaaactcactgatcttgaaaatctgcatcttcctctgcctctgctccagcccttgatgcagcaggtccctcagcctattcctcagactcttgcacttccccctcagcccctgtggtctgttcctcagcccaaagtcctgcctatcccccagcaagtggtgccctaccctcagagagctgtgcctgttcaagcccttctgctcaaccaagaacttctacttaaccccacccaccagatctaccctgtgactcagccacttgccccagttcataaccccattagtgtctaa

SEQ ID NO: 22 - DNA, 549 bp, human
atgaagagttttcttctagttgtcaatgccctggcattaaccctgccttttttggctgtggaggttcaaaaccagaaacaaccagcatgccatgagaatgatgaaagaccattctatcagaaaacagctccatatgtcccaatgtattatgtgccaaatagctatccttattatggaaccaatttgtaccaacgtagaccagctatagcaattaataatccatatgtgcctcgcacatattatgcaaacccagctgtagttaggccacatgcccaaattcctcagcggcaatacctgccaaatagccacccacccactgtggtacgtcgcccaaacctgcatccatcatttattgccatccccccaaagaaaattcaggataaaataatcatccctaccatcaataccattgctactgttgaacctacaccagctcctgccactgaaccaacggtggacagtgtagtcactccagaagctttttcagagtccatcatcacgagcacccctgagacaaccacagttgcagttactccacctacggcataa

SEQ ID NO: 23 - protein, 584 aa, human
MKMMLVRRFRVLILMVFLVACALHIALDLLPRLERRGARPSGEPGCSCAQPAAEVAAPGWAQVRGRPGEPPAASSAAGDAGWPNKHTLRILQDFSSDPSSNLSSHSLEKLPPAAEPAERALRGRDPGALRPHDPAHRPLLRDPGPRRSESPPGPGGDASLLARLFEHPLYRVAVPPLTEEDVLFNVNSDTRLSPKAAENPDWPHAGAEGAEFLSPGEAAVDSYPNWLKFHIGINRYELYSRHNPAIEALLHDLSSQRITSVAMKSGGTQLKLIMTFQNYGQALFKPMKQTREQETPPDFFYFSDYERHNAEIAAFHLDRILDFRRVPPVAGRMVNMTKEIRDVTRDKKLWRTFFISPANNICFYGECSYYCSTEHALCGKPDQIEGSLAAFLPDLSLAKRKTWRNPWRRSYHKRKKAEWEVDPDYCEEVKQTPPYDSSHRILDVMDMTIFDFLMGNMDRHHYETFEKFGNETFIIHLDNGRGFGKYSHDELSILVPLQQCCRIRKSTYLRLQLLAKEEYKLSLLMAESLRGDQVAPVLYQPHLEALDRRLRVVLKAVRDCVERNGLHSVVDDDLDTEHRAASAR

SEQ ID NO: 24 - DNA, 276 bp, artificial
  secretion signal
atgaggcaggtttggttctcttggattgtgggattgttcctatgttttttcaacgtgtcttctgctgctccagtcaacactacaacagaagatgaaacggcacaaattccggctgaagctgtcatcggttactcagatttagaaggggatttcgatgttgctgttttgccattttccaacagcacaaataacgggttattgtttataaatactactattgccagcattgctgctaaagaagaaggggtatctttggataaaagagaggctgaagct

SEQ ID NO: 25 - DNA, 267 bp, artificial
  secretion signal
atgaaattctctactatattagccgcatctactgctttaatttccgttgttatggctgctccagtttctaccgaaactgacatcgacgatcttccaatatcggttccagaagaagccttgattggattcattgacttaaccggggatgaagtttccttgttgcctgttaataacggaacccacactggtattctattcttaaacaccaccatcgctgaagctgctttcgctgacaaggatgatctcgagaaaagagaggctgaagct

SEQ ID NO: 26 - DNA, 57 bp, artificial
  secretion signal
atgagatttccttcaatttttactgctgttttattcgcagcatcctccgcattagct

SEQ ID NO: 27 - DNA, 78 bp, artificial
  signal sequence
atgactaagccaacccaagtattagttagatccgtcagtatattatttttcatcacattactacatctagtcgtagct

SEQ ID NO: 28 - DNA, 1637 bp, artificial
  promoter
gtcagtaccgactgggatcttggcagcttgaacggcatcagcagtagcgtattgttggaaagaaccgtcgtgagtgtaaccggacaagtcagcttctggacagttggattcgttggacaattcacagtattcacaggacatacaagaaccgttcaaccatttgataccagcgaagtcaccaatcttccagcccttgacgttttcacccatagcaacaacgacaccagcaccttcgtgaccaccaactaatggcaatttggttggcaaaggccagtcacccttccatgcgtgcaaatcggtgtgacagacaccggagtacttgacgttgatcaaaagttcgttagcctttggctttggaactgggatgtccttgtattgcaattcaccaccgttttcgtagaagataacacccttttgagtttctgggatagatgcggccattttatctttttttagtatagagtttgtgtgtttaaagcttgtttatgtttcaattgaaactattgtttttgcttgatgatgatgtagggcaaaacagaaacaacattgtacaaatggatatagagagacctactacaaaagtggatggattgtcagaatcgaccgggtgtttatatacatattccagaagaccaaatggctggtctaattgtatacaagtaagacagctgatttctagctggtgtgaaaatagcacactttgagaaaaatacataccaccctgcaacaggtgttaaccgtttaagacctagaaataaccgcagtatataaagatcaatcgaatacttgggttggtgaaaagcaacccaaaatacatcatctgctcatatgattgtgatctgattgtgaatagatcaatacactactagaatagaagaacatcacacgctatttttttttcctcttctgtcctactcggagaaacagaaagtatcaggtcaccaccggacatgtcatactatctagataatcgggtatgattaacagcgacatagctatgtgattatctgccccattacttaaagtaaggtttcactttcggactaaggacgaatgacacaagacacagaacgctcacacggttgaaacattttttttcctgatccttttgaccctgtttgttgtccctcttttacgatgggagaattgaatcatccgccattaaaccgaatgtgatagtttttccagtttttcttcccctccctacatccatttctaaagaattcacggacattttcgcatgaatggggaaagttgactcagttgactctatttggttcctcagcctcgactgctttgcttcatcttctctatgggccaatgagctaatgagcacaatgtgctgcgaaataaagggatatctaatttatattattacattataatatgtactagtgtggttattggtaattgtacttaattttgatatataaagggtggatctttttcattttgaatcagaattggaattgcaacttgtctcttgtcactattacttaatagtaattatatttcttattaaccttttttttaagtcaaaacaccaaggacaagaactactcttcaaaggtatttcaagttatcatacgtctcacacacgcttcacagtttcaagtaaaaaaaaagaatattacaca

SEQ ID NO: 29 - DNA, 60 bp, artificial
  linker 1
agagctgagggtagaggttctttgcttacttgcggtgacgttgaggaaaacccaggtcca

SEQ ID NO: 30 - DNA, 60 bp, artificial
  linker
cgtgccgaaggacgtggatcccttttgacctgcggagatgtcgaagagaatcctggacct

SEQ ID NO: 31 - DNA, 60 bp, artificial
  signal sequence
atggtcgcttggtggtctttgtttctgtacggtcttcaggtcgctgcacctgctttggct

SEQ ID NO: 32 - DNA, 54 bp, artificial
  signal sequence
atgtcttttagatccttgttggctttgtctggtttggtttgttctggtttggct

SEQ ID NO: 33 - DNA, 54 bp, artificial
  signal sequence
atgaagtgggttacctttatctctttgttgtttcttttctcttctgcttactct

SEQ ID NO: 34 - DNA, 48 bp, artificial
  signal sequence
atgaagttagcatactccttgttgcttccattggcaggagtcagtgct

SEQ ID NO: 35 - DNA, 57 bp, artificial
  signal sequence
atgcttttgcaagctttccttttccttttggctggttttgcagccaaaatatctgca

SEQ ID NO: 36 - DNA, 78 bp, artificial
  signal sequence
atgctgggtaagaacgacccaatgtgtcttgttttggtcttgttgggattgactgctttgttgggtatctgtcaaggt

SEQ ID NO: 37 - DNA, 939 bp, artificial
  promoter
gatctaacatccaaagacgaaaggttgaatgaaacctttttgccatccgacatccacaggtccattctcacacataagtgccaaacgcaacaggaggggatacactagcagcagaccgttgcaaacgcaggacctccactcctcttctcctcaacacccacttttgccatcgaaaaaccagcccagttattgggcttgattggagctcgctcattccaattccttctattaggctactaacaccatgactttattagcctgtctatcctggcccccctggcgaggttcatgtttgtttatttccgaatgcaacaagctccgcattacacccgaacatcactccagatgagggctttctgagtgtggggtcaaatagtttcatgttccccaaatggcccaaaactgacagtttaaacgctgtcttggaacctaatatgacaaaagcgtgatctcatccaagatgaactaagtttggttcgttgaaatgctaacggccagttggtcaaaaagaaacttccaaaagtcggcataccgtttgtcttgtttggtattgattgacgaatgctcaaaaataatctcattaatgcttagcgcagtctctctatcgcttctgaaccccggtgcacctgtgccgaaacgcaaatggggaaacacccgctttttggatgattatgcattgtctccacattgtatgcttccaagattctggtgggaatactgctgatagcctaacgttcatgatcaaaatttaactgttctaacccctacttgacagcaatatataaacagaaggaagctgccctgtcttaaacctttttttttatcatcattattagcttactttcataattgcgactggttccaattgacaagcttttgattttaacgacttttaacgacaacttgagaagatcaaaaaacaactaattattcgaaacg